European Patent Specification EP 3 777 879 B1, published September 3, 2025. Title: COMPOSITIONS AND METHODS FOR TREATING HEART FAILURE. Applicant: ZENSUN (SHANGHAI) SCIENCE AND TECHNOLOGY, Co., Ltd. Application Divisional application based on EP 16183775.2. The sequence listing filed with the application follows.

SEQUENCE LISTING (2 sequences)

SEQ ID NO: 1 - protein, 61 aa, Homo sapiens
SHLVKCAEKEKTFCVNGGECFMVKDLSNPSRYLCKCPNEFTGDRCQNYVMASFYKAEELYQ

SEQ ID NO: 2 - protein, 23 aa, Homo sapiens
AEKEKTFCVNGGECFMVKDLSNP